European Patent Application EP 4 257 612 A1, published October 11, 2023. Title: Development of new tumor engager therapeutic drug and use thereof. Applicant: Keymed Biosciences Co.,Ltd. The sequence listing filed with the application follows.

SEQUENCE LISTING (173 sequences)

SEQ ID NO: 1 - protein, 552 aa, Homo sapiens
QPPPPPPDATCHQVRSFFQRLQPGLKWVPETPVPGSDLQVCLPKGPTCCSRKMEEKYQLTARLNMEQLLQSASMELKFLIIQNAAVFQEAFEIVVRHAKNYTNAMFKNNYPSLTPQAFEFVGEFFTDVSLYILGSDINVDDMVNELFDSLFPVIYTQLMNPGLPDSALDINECLRGARRDLKVFGNFPKLIMTQVSKSLQVTRIFLQALNLGIEVINTTDHLKFSKDCGRMLTRMWYCSYCQGLMMVKPCGGYCNVVMQGCMAGVVEIDKYWREYILSLEELVNGMYRIYDMENVLLGLFSTIHDSIQYVQKNAGKLTTTIGKLCAHSQQRQYRSAYYPEDLFIDKKVLKVAHVEHEETLSSRRRELIQKLKSFISFYSALPGYICSHSPVAENDTLCWNGQELVERYSQKAARNGMKNQFNLHELKMKGPEPVVSQIIDKLKHINQLLRTMSMPKGRVLDKNLDEEGFESGDCGDDEDECIGGSGDGMIKVKNQLRFLAELAYDLDVDDAPGNSQQATPKDNEISTFHNLGNVHSPLKASGGGGSHHHHHH

SEQ ID NO: 2 - protein, 218 aa, Homo sapiens
MSPILGYWKIKGLVQPTRLLLEYLEEKYEEHLYERDEGDKWRNKKFELGLEFPNLPYYIDGDVKLTQSMAIIRYIADKHNMLGGCPKERAEISMLEGAVLDIRYGVSRIAYSKDFETLKVDFLSKLPEMLKMFEDRLCHKTYLNGDHVTHPDFMLYDALDVVLYMDPMCLDAFPKLVCFKKRIEAIPQIDKYLKSSKYIAWPLQGWQATFGGGDHPPK

SEQ ID NO: 3 - protein, 282 aa, Macaca fascicularis
MSPILGYWKIKGLVQPTRLLLEYLEEKYEEHLYERDEGDKWRNKKFELGLEFPNLPYYIDGDVKLTQSMAIIRYIADKHNMLGGCPKERAEISMLEGAVLDIRYGVSRIAYSKDFETLKVDFLSKLPEMLKMFEDRLCHKTYLNGDHVTHPDFMLYDALDVVLYMDPMCLDAFPKLVCFKKRIEAIPQIDKYLKSSKYIAWPLQGWQATFGGGDHPPKSDLIEGRGIPGAELAYDLDVDDVPGNNQQATPKDNEISTFHNLGNVHSPLKASGGGGSHHHHHH

SEQ ID NO: 4 - protein, 282 aa, Mus musculus
MSPILGYWKIKGLVQPTRLLLEYLEEKYEEHLYERDEGDKWRNKKFELGLEFPNLPYYIDGDVKLTQSMAIIRYIADKHNMLGGCPKERAEISMLEGAVLDIRYGVSRIAYSKDFETLKVDFLSKLPEMLKMFEDRLCHKTYLNGDHVTHPDFMLYDALDVVLYMDPMCLDAFPKLVCFKKRIEAIPQIDKYLKSSKYIAWPLQGWQATFGGGDHPPKSDLIEGRGIPGAELAYDLDVDDAPGNKQHGNQKDNEITTSHSVGNMPSPLKASGGGGSHHHHHH

SEQ ID NO: 5 - protein, 306 aa, Homo sapiens
QSIKGNHLVKVYDYQEDGSVLLTCDAEAKNITWFKDGKMIGFLTEDKKKWNLGSNAKDPRGMYQCKGSQNKSKPLQVYYRMCQNCIELNAPEAAGGPSVFLFPPKPKDTLMISRTPEVTCVVVDVSHEDPEVKFNWYVDGVEVHNAKTKPREEQYNSTYRVVSVLTVLHQDWLNGKEYKCKVSNKALPASIEKTISKAKGQPREPQVCTLPPSRDELTKNQVSLSCAVKGFYPSDIAVEWESNGQPENNYKTTPPVLDSDGSFFLVSKLTVDKSRWQQGNVFSCSVMHEALHNHYTQKSLSLSPGK

SEQ ID NO: 6 - protein, 339 aa, Homo sapiens
QDGNEEMGGITQTPYKVSISGTTVILTCPQYPGSEILWQHNDKNIGGDEDDKNIGSDEDHLSLKEFSELEQSGYYVCYPRGSKPEDANFYLYLRARVCENCMEMDAPEAAGGPSVFLFPPKPKDTLMISRTPEVTCVVVDVSHEDPEVKFNWYVDGVEVHNAKTKPREEQYNSTYRVVSVLTVLHQDWLNGKEYKCKVSNKALPASIEKTISKAKGQPREPQVYTLPPCRDELTKNQVSLWCLVKGFYPSDIAVEWESNGQPENNYKTTPPVLDSDGSFFLYSKLTVDKSRWQQGNVFSCSVMHEALHNHYTQKSLSLSPGKGSGLNDIFEAQKIEWHE

SEQ ID NO: 7 - protein, 305 aa, Macaca fascicularis
QSFEENRKLNVYNQEDGSVLLTCHVKNTNITWFKEGKMIDILTAHKNKWNLGSNTKDPRGVYQCKGSKDKSKTLQVYYRMCQNCIELNAPEAAGGPSVFLFPPKPKDTLMISRTPEVTCVVVDVSHEDPEVKFNWYVDGVEVHNAKTKPREEQYNSTYRVVSVLTVLHQDWLNGKEYKCKVSNKALPASIEKTISKAKGQPREPQVCTLPPSRDELTKNQVSLSCAVKGFYPSDIAVEWESNGQPENNYKTTPPVLDSDGSFFLVSKLTVDKSRWQQGNVFSCSVMHEALHNHYTQKSLSLSPGK

SEQ ID NO: 8 - protein, 330 aa, Macaca fascicularis
QDGNEEMGSITQTPYQVSISGTTVILTCSQHLGSEAQWQHNGKNKEDSGDRLFLPEFSEMEQSGYYVCYPRGSNPEDASHHLYLKARVCENCMEMDAPEAAGGPSVFLFPPKPKDTLMISRTPEVTCVVVDVSHEDPEVKFNWYVDGVEVHNAKTKPREEQYNSTYRVVSVLTVLHQDWLNGKEYKCKVSNKALPASIEKTISKAKGQPREPQVYTLPPCRDELTKNQVSLWCLVKGFYPSDIAVEWESNGQPENNYKTTPPVLDSDGSFFLYSKLTVDKSRWQQGNVFSCSVMHEALHNHYTQKSLSLSPGKGSGLNDIFEAQKIEWHE

SEQ ID NO: 9 - protein, 115 aa, Mus musculus
QVQLQQSGAELVRPGASVKLSCKALGYTFADYEIHWVKQTPVHGLEWIGAIHPGSGGTAYNQTFEGKATLTADKSSTTAYMELSSLTSEDSAVYYCTRYYSFAYWGQGTLVTVSA

SEQ ID NO: 10 - DNA, 345 bp, Mus musculus
caggtccagctgcagcagtctggggctgagctggtgaggcctggggcttcagtgaagctgtcctgcaaggctttgggctacacatttgctgactatgaaatacactgggtgaagcagacacctgtgcatggcctggagtggattggagctattcatccaggaagtggtggtactgcctacaatcagacgttcgagggcaaggccacactgactgcagacaaatcctccaccacagcctacatggagctcagcagcctgacatctgaggactctgctgtctattactgtacaagatactattcctttgcttactggggccaagggactctggtcactgtctctgca

SEQ ID NO: 11 - protein, 6 aa, Mus musculus
ADYEIH

SEQ ID NO: 12 - protein, 17 aa, Mus musculus
AIHPGSGGTAYNQTFEG

SEQ ID NO: 13 - protein, 6 aa, Mus musculus
YYSFAY

SEQ ID NO: 14 - protein, 112 aa, Mus musculus
DVLMTQTPLSLPVSLGDQASISCRSSQSLVHSNGNTYLHWYLQKPGQSPKLLIYKVSNRFSGVPDRFSGSGSGTDFTLKISRVEAEDLGVYFCSQSTHVPLTFGAGTKLELK

SEQ ID NO: 15 - DNA, 336 bp, Mus musculus
gatgttttgatgacccaaactccactctccctgcctgtcagtcttggagatcaagcctccatctcttgcagatctagtcagagccttgtacacagtaatggaaacacctatttacattggtacctgcagaagccaggccagtctccaaagctcctgatctacaaagtttccaaccgattttctggggtcccagacaggttcagtggcagtggatcagggacagatttcacactcaagatcagcagagtggaggctgaggatctgggagtttatttctgctctcaaagtacacatgttccgctcacgttcggtgctgggaccaagctggagctgaaa

SEQ ID NO: 16 - protein, 16 aa, Mus musculus
RSSQSLVHSNGNTYLH

SEQ ID NO: 17 - protein, 7 aa, Mus musculus
KVSNRFS

SEQ ID NO: 18 - protein, 9 aa, Mus musculus
SQSTHVPLT

SEQ ID NO: 19 - protein, 115 aa, Mus musculus
EVQLQQSGAELVRPGASVKLSCKALGYTFADYEIHWVKQTPVHGLEWIGAIHPGSGGTAYNQTFKGKATLTADKSSTTAYMELSSLTSEDSAVYYCTRYYSFAYWGQGTLVTVSA

SEQ ID NO: 20 - DNA, 345 bp, Mus musculus
gaggttcaactgcagcagtctggggctgagctggtgaggcctggggcttcagtgaagctgtcctgcaaggctttgggctacacatttgctgactatgaaatacactgggtgaagcagacacctgtgcatggcctggagtggattggagctattcatccaggaagtggtggtactgcctacaatcagacgttcaagggcaaggccacactgactgcagacaaatcctccaccacagcctacatggagctcagcagcctgacatctgaggactctgctgtctattactgtacaagatactattcctttgcttactggggccaagggactctggtcactgtctctgca

SEQ ID NO: 21 - protein, 17 aa, Mus musculus
AIHPGSGGTAYNQTFKG

SEQ ID NO: 22 - protein, 112 aa, Mus musculus
DVVMTQTPLSLPVSLGDQASISCRSSQSLVHSNGNTYLHWYLQKPGQSPKLLIYKVSNRFSGVPDRFSGSGSGTDFTLKISRVEAEDLGVYFCSQSTHVPLTFGAGTKLEIK

SEQ ID NO: 23 - DNA, 336 bp, Mus musculus
gatgttgtgatgacccaaactccactctccctgcctgtcagtcttggagatcaagcctccatctcttgcagatctagtcagagccttgtacacagtaatggaaacacctatttacattggtacctgcagaagccaggccagtctccaaagctcctgatctacaaagtttccaaccgattttctggggtcccagacaggttcagtggcagtggatcagggacagatttcacactcaagatcagcagagtggaggctgaggatctgggagtttatttctgctctcaaagtacacatgttccgctcacgttcggtgctgggaccaagctggaaataaaa

SEQ ID NO: 24 - protein, 112 aa, Mus musculus
DVVMTQTPLSLPVSLGDQASISCRSSQSLVHSNGNTYLHWYLQKPGQSPKLLIYKVSNRFSGVPDRFSGSGSGTDFTLKISRVEAEDLGVYFCSQSIHVPLTFGAGTKLELK

SEQ ID NO: 25 - DNA, 336 bp, Mus musculus
gatgttgtgatgacccaaactccactctccctgcctgtcagtcttggagatcaagcctccatctcttgcagatctagtcagagccttgtacacagtaatggaaacacctatttacattggtacctgcagaagccaggccagtctccaaagctcctgatctacaaagtttccaaccgattttctggggtcccagacaggttcagtggcagtggatcagggacagatttcacactcaagatcagcagagtggaggctgaggatctgggagtttatttctgctctcaaagtatacatgttccgctcacgttcggtgctgggaccaagctggagctgaaa

SEQ ID NO: 26 - protein, 9 aa, Mus musculus
SQSIHVPLT

SEQ ID NO: 27 - protein, 111 aa, Mus musculus
DVLMTQTPLSLPVSLGDQASISCRSSQSLVHSNGNTYLHWYLQKPGQSPKLLIYKVSNRFSGVPDRFSGSGSGTDFTLKISRVEAEDLGVYFCSQSTHIPTFGGGTKLELK

SEQ ID NO: 28 - DNA, 333 bp, Mus musculus
gatgttttgatgacccaaactccactctccctgcctgtcagtcttggagatcaagcctccatctcttgcagatctagtcagagccttgtacacagtaatggaaacacctatttacattggtacctgcagaagccaggccagtctccaaagctcctgatctacaaagtttccaaccgattttctggggtcccagacaggttcagtggcagtggatcagggacagatttcacactcaagatcagcagagtggaggctgaggatctgggagtttatttctgctctcaaagtacacatattcccacgttcggtggaggcaccaagctggagctgaaa

SEQ ID NO: 29 - protein, 8 aa, Mus musculus
SQSTHIPT

SEQ ID NO: 30 - protein, 115 aa, Mus musculus
QVQLQQSGAELVRPGASVRLSCKALGYTFTDYEMHWVKQTPVHGLEWIGAIHPGSGGTAYNQKFKGKATLTADKSSSTAYMELSSLTSEDSAVYYCTRYYSFAYWGQGTLVTVSA

SEQ ID NO: 31 - DNA, 345 bp, Mus musculus
caggttcagctgcagcagtctggggctgagctggtgaggcctggggcttcagtgaggctgtcctgcaaggctttgggctacacatttactgactatgaaatgcactgggtgaagcagacacctgtgcatggcctggaatggattggagctattcatccaggaagtggtggtactgcctacaatcagaagttcaagggcaaggccacactgactgcagacaaatcctccagcacagcctacatggagctcagcagcctgacatctgaggactctgctgtctattactgtacaagatactattcctttgcttactggggccaagggactctggtcactgtctctgca

SEQ ID NO: 32 - protein, 6 aa, Mus musculus
TDYEMH

SEQ ID NO: 33 - protein, 17 aa, Mus musculus
AIHPGSGGTAYNQKFKG

SEQ ID NO: 34 - protein, 112 aa, Mus musculus
DVLMTQTPLSLPVSLGDQASISCRSSQSLVHSNGNTYLHWYLQKPGQSPKLLIYKVSNRFSGVPDRFSGSGSGTDFTLKISRVEAEDLGVYFCSQSTHVPLTFGAGTKLEIK

SEQ ID NO: 35 - DNA, 336 bp, Mus musculus
gatgttttgatgacccaaactccactctccctgcctgtcagtcttggagatcaagcctccatctcttgcagatctagtcagagccttgtacacagtaatggaaacacctatttacattggtacctgcagaagccaggccagtctccaaagctcctgatctacaaagtttccaaccgattttctggggtcccagacaggttcagtggcagtggatcagggacagatttcacactcaagatcagcagagtggaggctgaggatctgggagtttatttctgctctcaaagtacacatgttccgctcacgttcggtgctgggaccaagctggaaatcaaa

SEQ ID NO: 36 - protein, 112 aa, Mus musculus
DVLMTQTPLSLPVSLGDQASISCRSSQSIVHSNGNTYLQWYLQKPGQSPKLLIYKVSNRFSGVPDRFSGSGSGTDFTLKISRVEAEDLGVYYCFQGSHVPYTFGGGTKLEIK

SEQ ID NO: 37 - DNA, 336 bp, Mus musculus
gatgttttgatgacccaaactccactctccctgcctgtcagtcttggagatcaagcctccatctcttgcagatctagtcagagcattgtacatagtaatggaaacacctatttacaatggtacctgcagaaaccaggccagtctccaaagctcctgatctacaaagtttccaaccgattttctggggtcccagacaggttcagtggcagtggatcagggacagatttcacactcaagatcagcagagtggaggctgaggatctgggagtttattactgctttcaaggttcacatgttccgtacacgttcggaggggggaccaagctggaaataaaa

SEQ ID NO: 38 - protein, 16 aa, Mus musculus
RSSQSIVHSNGNTYLQ

SEQ ID NO: 39 - protein, 9 aa, Mus musculus
FQGSHVPYT

SEQ ID NO: 40 - protein, 115 aa, Mus musculus
QVQLQQSGAELVRPGASVKLSCKALGYAFADYEIHWVKQTPVHGLEWIGAIHPGSGGTAYNQTFKGKATLTADKSSTTAYMELSSLTSEDSAVYYCTRYYSFAYWGQGTLVTVSA

SEQ ID NO: 41 - DNA, 345 bp, Mus musculus
caggtccagctgcagcagtctggggctgagctggtgaggcctggggcttcagtgaagctgtcctgcaaggctttgggctacgcatttgctgactatgaaatacactgggtgaagcagacacctgtgcatggcctggagtggattggagctattcatccaggaagtggtggtactgcctacaatcagacgttcaagggcaaggccacactgactgcagacaaatcctccaccacagcctacatggagctcagcagcctgacatctgaggactctgctgtctattactgtacaagatactattcctttgcttactggggccaagggactctggtcactgtctctgca

SEQ ID NO: 42 - protein, 112 aa, Mus musculus
DVVMTQTPLSLPVSLGDQASISCRSSQSLVHSNGNTYLHWYLQKPGQSPKLLIYKVSNRFSGVPDRFSGSGSGTDFTLKISRVEAEDLGVYFCSQSTHVPLTFGAGTKLELK

SEQ ID NO: 43 - DNA, 336 bp, Mus musculus
gatgttgtgatgacccaaactccactctccctgcctgtcagtcttggagatcaagcctccatctcttgcagatctagtcagagccttgtacacagtaatggaaacacctatttacattggtacctgcagaagccaggccagtctccaaagctcctgatctacaaagtttccaaccgattttctggggtcccagacaggttcagtggcagtggatcagggacagatttcacactcaagatcagcagagtggaggctgaggatctgggagtttatttctgctctcaaagtacacatgttccgctcacgttcggtgctgggaccaagctggagctgaaa

SEQ ID NO: 44 - protein, 112 aa, Mus musculus
DVVMTQTPLSLPVSLGDQASISCRSSQSLENSNGNTYLNWYLQKPGQSPQLLIYRVSNRFSGVLDRFSGSGSGTDFTLKISRVEAEDLGVYFCLQVTHVPYTFGGGTKLEIK

SEQ ID NO: 45 - DNA, 336 bp, Mus musculus
gatgttgtgatgacccaaactccactctccctgcctgtcagtcttggagatcaagcctccatctcttgcaggtctagtcagagccttgaaaacagtaatggaaacacctatttgaactggtacctccagaaaccaggccagtctccacagctcctgatctacagggtttccaaccgattttctggggtcctagacaggttcagtggtagtggatcagggacagatttcacactgaaaatcagcagagtggaggctgaggatttgggagtttatttctgcctccaagttacacatgtcccgtacacgttcggaggggggaccaagctggaaataaaa

SEQ ID NO: 46 - protein, 16 aa, Mus musculus
RSSQSLENSNGNTYLN

SEQ ID NO: 47 - protein, 7 aa, Mus musculus
RVSNRFS

SEQ ID NO: 48 - protein, 9 aa, Mus musculus
LQVTHVPYT

SEQ ID NO: 49 - protein, 111 aa, Mus musculus
DVVVTQTPLSLPVSLGDQASISCRSSQSLVHSNGNTYLHWYLQKPGQSPKLLIYKVSNRFSGVPDRFSGSGSGTDFTLKISRVEAEDLGVYFCSQSTHVPTFGGGTKLEIK

SEQ ID NO: 50 - DNA, 333 bp, Mus musculus
gatgttgtggtgactcaaactccactctccctgcctgtcagtcttggagatcaggcctccatctcttgcagatctagtcagagccttgtacacagtaatggaaacacctatttacattggtacctgcagaagccaggccagtctccaaagctcctgatctacaaagtttccaaccgattttctggggtcccagacaggttcagtggcagtggatcagggacagatttcacactcaagatcagcagagtggaggctgaggatctgggagtttatttctgctctcaaagtacacatgttccgacgttcggtggaggcaccaagctggaaatcaaa

SEQ ID NO: 51 - protein, 8 aa, Mus musculus
SQSTHVPT

SEQ ID NO: 52 - protein, 112 aa, Mus musculus
DVLMTQTPLSLPVSLGDQASISCRSSQSLVHSNGNTYLHWYLQKPGQSPKLLIYKVSNRFSGVPDRFSGSGSGTDFTLKISRVEAEDLGVYFCSQNTHVPLTFGAGTKLELK

SEQ ID NO: 53 - DNA, 336 bp, Mus musculus
gatgttttgatgacccaaactccactctccctgcctgtcagtcttggagatcaagcctccatctcttgcagatctagtcagagccttgtacacagtaatggaaacacctatttacattggtacctgcagaagccaggccagtctccaaagctcctgatctacaaagtttccaaccgattttctggggtcccagacaggttcagtggcagtggatcagggacagatttcacactcaagatcagcagagtggaggctgaggatctgggagtttatttctgctctcaaaatacacatgttccgctcacgttcggtgctgggaccaagctggagctgaaa

SEQ ID NO: 54 - protein, 9 aa, Mus musculus
SQNTHVPLT

SEQ ID NO: 55 - protein, 112 aa, Mus musculus
DVVMTQTPLSLPVSLGDQASISCRSSQSLVHSNGNTYLHWYLQKPGQSPKLLIYKVSNRFSGVPDRFSGSGSGTDFTLRISRVEAEDLGVYFCSQSTRVPLTFGAGTKLELK

SEQ ID NO: 56 - DNA, 336 bp, Mus musculus
gatgttgtgatgacccagactccactctccctgcctgtcagtcttggagatcaagcctccatctcttgcagatctagtcagagccttgtacacagtaatggaaacacctatttacattggtacctgcagaagccaggccagtctccaaagctcctgatctacaaagtttccaaccgattttctggggtcccagacaggttcagtggcagtggatcagggacagatttcacactcaggatcagcagagtggaggctgaggatctgggagtttatttctgctctcaaagtacacgtgttccgctcacgttcggtgctgggaccaagctggagctgaaa

SEQ ID NO: 57 - protein, 9 aa, Mus musculus
SQSTRVPLT

SEQ ID NO: 58 - protein, 112 aa, Mus musculus
DVVMTQTPLSLPVSLGDQASISCRSSQSIVHSNGNTYLEWYLQKPGQSPKLLIYKVSNRFSGVPDRFSGSGSGTDFTLKISRVEAEDLGVYFCLQVTHVPLTFGAGTKLELK

SEQ ID NO: 59 - DNA, 336 bp, Mus musculus
gatgttgtgatgacccaaactccactctccctgcctgtcagtcttggagatcaagcctccatctcttgcagatctagtcagagcattgtacatagtaatggaaacacctatttagaatggtacctgcagaaaccaggccagtctccaaagctcctgatctacaaagtttccaaccgattttctggggtcccagacaggttcagtggcagtggatcagggacagatttcacactcaagatcagcagagtggaggctgaggatctgggagtttatttctgcctccaagttacacatgtcccgctcacgttcggtgctgggaccaagctggagctgaaa

SEQ ID NO: 60 - protein, 16 aa, Mus musculus
RSSQSIVHSNGNTYLE

SEQ ID NO: 61 - protein, 9 aa, Mus musculus
LQVTHVPLT

SEQ ID NO: 62 - protein, 111 aa, Mus musculus
QVQLQQSGPELVKPGASVKISCKASGYTFTDYYINWVKQKPGQGLEWIGWIYPGSGNTKYNEKFKGKATLTVDTSSSTAYMQLSSLTSEDTAVYFCARGRWGQGTLVTVSA

SEQ ID NO: 63 - DNA, 333 bp, Mus musculus
caggtccagttgcaacagtctggacctgagctggtgaagcctggggcttcagtgaagatatcctgcaaggcttctggctacaccttcactgactactatataaactgggtgaagcagaagcctggacagggacttgagtggattggatggatttatcctggaagcggtaatactaagtacaatgagaagttcaagggcaaggccacattgactgtagacacatcctccagcacagcctacatgcagctcagcagcctgacatccgaggacactgctgtctatttctgtgcaagggggcgctggggccaagggactctggtcactgtctctgca

SEQ ID NO: 64 - protein, 6 aa, Mus musculus
TDYYIN

SEQ ID NO: 65 - protein, 17 aa, Mus musculus
WIYPGSGNTKYNEKFKG

SEQ ID NO: 66 - protein, 2 aa, Mus musculus
GR

SEQ ID NO: 67 - protein, 112 aa, Mus musculus
DVVMTQTPLSLPVSLRDQASISCRSSQSLVHSNGNTYLHWYLQKPGQSPKLLIYKVSNRFSGVPDRFSGSGSGTDFTLKISRVEAEDLGVYFCSQSTHVPRTFGGGTKLELK

SEQ ID NO: 68 - DNA, 336 bp, Mus musculus
gatgttgtgatgacccagactccactctccctgcctgtcagtcttcgagatcaagcctccatctcttgcagatctagtcagagccttgtacacagtaatggaaacacctatttacattggtacctgcagaagccaggccagtctccaaagctcctgatctacaaagtttccaaccgattttctggggtcccagacaggttcagtggcagtggatcagggacagatttcacactcaagatcagcagagtggaggctgaggatctgggagtttatttctgctctcaaagtacacatgttcctcggacgttcggtggaggcaccaagctggagctgaaa

SEQ ID NO: 69 - protein, 9 aa, Mus musculus
SQSTHVPRT

SEQ ID NO: 70 - protein, 115 aa, Mus musculus
QVQLQQSGAELVRPGASVKLSCKALGYTFADYEIHWVKQTPVHGLEWIGAIHPGSGGTAYSQTFKGKATLTADKSSTTAYMELSSLTSEDSAVYYCTRYFSFAYWGQGTLVTVSA

SEQ ID NO: 71 - DNA, 345 bp, Mus musculus
caggttcagctgcagcagtctggggctgagctggtgaggcctggggcttcagtgaagctgtcctgcaaggctttgggctacacatttgctgactatgaaatacactgggtgaagcagacacctgtgcatggcctggaatggattggagctattcatccaggaagtggtggtactgcctacagtcagacgttcaagggcaaggccacactgactgcagacaaatcctccaccacagcctacatggagctcagcagcctgacatctgaggactctgctgtctattactgtacaagatacttttcctttgcttactggggccaagggactctggtcactgtctctgca

SEQ ID NO: 72 - protein, 17 aa, Mus musculus
AIHPGSGGTAYSQTFKG

SEQ ID NO: 73 - protein, 6 aa, Mus musculus
YFSFAY

SEQ ID NO: 74 - protein, 112 aa, Mus musculus
DVVVTQTPLSLPVSLGDQASISCRSSQSLVHSNGNTYLHWYLQKPGQSPKLLIYKVSNRFSGVPDRFSGSGSGTDFTLKISRVEAEDLGVYFCSQSTHAPYTFGGGTRLEIK

SEQ ID NO: 75 - DNA, 336 bp, Mus musculus
gatgttgtggtgactcaaactccactctccctgcctgtcagtcttggagatcaagcctccatctcttgcagatctagtcagagccttgtacacagtaatggaaacacctatttacattggtacctgcagaagccaggccagtctccaaagctcctgatctacaaagtttccaaccgattttctggggtcccagacaggttcagtggcagtggatcagggacagatttcacactcaagatcagcagagtggaggctgaggatctgggagtttatttctgctctcaaagtacacatgctccgtacacgttcggaggggggaccagactggaaataaaa

SEQ ID NO: 76 - protein, 9 aa, Mus musculus
SQSTHAPYT

SEQ ID NO: 77 - protein, 111 aa, Mus musculus
QVQLQQSGAELMKPGASVKISCKATGYTFSSYWIEWVKQRPGHGLEWIGEILPGSGSTNYNEKFKGKATFTADTSSNTAYMQLSSLTSEDSAVYYCARGYWGQGTLVTVSA

SEQ ID NO: 78 - DNA, 333 bp, Mus musculus
caggttcagctgcaacagtctggagctgagctgatgaagcctggggcctcagtgaagatatcctgcaaggctactggctacacattcagtagctactggatagagtgggtaaagcagaggcctggacatggccttgagtggattggagagattttacctggaagtggtagtactaactacaatgagaagttcaagggcaaggccacattcactgcagatacatcctccaacacagcctacatgcaactcagcagcctgacatctgaggactctgccgtctattactgtgcgaggggttactggggccaagggactctggtcactgtctctgca

SEQ ID NO: 79 - protein, 6 aa, Mus musculus
SSYWIE

SEQ ID NO: 80 - protein, 17 aa, Mus musculus
EILPGSGSTNYNEKFKG

SEQ ID NO: 81 - protein, 2 aa, Mus musculus
GY

SEQ ID NO: 82 - protein, 112 aa, Mus musculus
DIVMTQAPLSLPVSLGDQASISCRSSQSLVHSNGNTYLHWYLQKPGQSPKLLIYKVSNRFSGVPDRFSGSGSGTDFTLKISRVEAEDLGVYFCSQSTHVPRTFGGGTKLEIK

SEQ ID NO: 83 - DNA, 336 bp, Mus musculus
gatattgtgatgacgcaggctccactctccctgcctgtcagtcttggagatcaagcctccatctcttgcagatctagtcagagccttgtacacagtaatggaaacacctatttacattggtacctgcagaagccaggccagtctccaaagctcctgatctacaaagtttccaaccgattttctggggtcccagacaggttcagtggcagtggatcagggacagatttcacactcaagatcagcagagtggaggctgaggatctgggagtttatttctgctctcaaagtacacatgttcctcggacgttcggtggaggcaccaagctggaaatcaaa

SEQ ID NO: 84 - protein, 112 aa, Homo sapiens
DVVMTQSPLSLPVTLGQPASISCRSSQSIVHSNYNTYLEWYQQRPGQSPRLLIYKVSNRFSGVPDRFSGSGSGTDFTLKISRVEAEDVGVYFCLQVTHVPLTFGQGTKLEIK

SEQ ID NO: 85 - DNA, 336 bp, Homo sapiens
gacgtggtcatgacacagagccctctgagcctgcctgtgacactgggacagcctgccagcatcagctgtagaagcagccagagcatcgtgcacagcaactacaacacatacctggaatggtatcagcagaggcctggccagtctcctagactgctgatctacaaggtgtccaacagattcagcggcgtgcccgacagattctctggctctggatctggcaccgacttcaccctgaagatctccagagtggaagccgaggacgtgggcgtgtacttctgtctccaggtcacacacgtgcccctgacatttggccagggcaccaagctggaaatcaag

SEQ ID NO: 86 - protein, 112 aa, Homo sapiens
DVVMTQSPLSLPVTPGEPASISCRSSQSIVHSNYNTYLEWYLQKPGQSPQLLIYKVSNRFSGVPDRFSGSGSGTDFTLKISRVEAEDVGVYFCLQVTHVPLTFGQGTKLEIK

SEQ ID NO: 87 - DNA, 336 bp, Homo sapiens
gacgtggtcatgacacagagccctctgagcctgcctgtgacacctggcgaacctgccagcatcagctgtagaagcagccagagcatcgtgcacagcaactacaacacatacctggagtggtatctgcagaagcccggccagtctcctcagctgctgatctacaaggtgtccaacagattcagcggcgtgcccgacagattctctggctctggatctggcaccgacttcaccctgaagatctccagagtggaagccgaggacgtgggcgtgtacttctgtctccaggtcacacacgtgcccctgacatttggccagggcaccaagctggaaatcaag

SEQ ID NO: 88 - protein, 112 aa, Homo sapiens
DVVMTQSPLSLPVTPGEPASISCRSSQSIVHSNGNTYLEWYLQKPGQSPQLLIYKVSNRFSGVPDRFSGSGSGTDFTLKISRVEAEDVGVYFCLQVTHVPLTFGQGTKLEIK

SEQ ID NO: 89 - DNA, 336 bp, Homo sapiens
gacgtggtcatgacacagagccctctgagcctgcctgtgacacctggcgaacctgccagcatcagctgtagaagcagccagagcatcgtgcacagcaacggcaacacatacctggagtggtatctgcagaagcccggccagtctcctcagctgctgatctacaaggtgtccaacagattcagcggcgtgcccgacagattctctggctctggatctggcaccgacttcaccctgaagatctccagagtggaagccgaggacgtgggcgtgtacttctgtctccaggtcacacacgtgcccctgacatttggccagggcaccaagctggaaatcaag

SEQ ID NO: 90 - protein, 112 aa, Homo sapiens
DVVMTQSPLSLPVTPGEPASISCRSSQSIVHSNSNTYLEWYLQKPGQSPQLLIYKVSNRFSGVPDRFSGSGSGTDFTLKISRVEAEDVGVYFCLQVTHVPLTFGQGTKLEIK

SEQ ID NO: 91 - DNA, 336 bp, Homo sapiens
gacgtggtcatgacacagagccctctgagcctgcctgtgacacctggcgaacctgccagcatcagctgtagaagcagccagagcatcgtgcacagcaacagcaacacatacctggagtggtatctgcagaagcccggccagtctcctcagctgctgatctacaaggtgtccaacagattcagcggcgtgcccgacagattctctggctctggatctggcaccgacttcaccctgaagatctccagagtggaagccgaggacgtgggcgtgtacttctgtctccaggtcacacacgtgcccctgacatttggccagggcaccaagctggaaatcaag

SEQ ID NO: 92 - protein, 16 aa, Homo sapiens
RSSQSIVHSNSNTYLE

SEQ ID NO: 93 - protein, 112 aa, Homo sapiens
DVVMTQSPLSLPVTPGEPASISCRSSQSIVHSNTNTYLEWYLQKPGQSPQLLIYKVSNRFSGVPDRFSGSGSGTDFTLKISRVEAEDVGVYFCLQVTHVPLTFGQGTKLEIK

SEQ ID NO: 94 - DNA, 336 bp, Homo sapiens
gacgtggtcatgacacagagccctctgagcctgcctgtgacacctggcgaacctgccagcatcagctgtagaagcagccagagcatcgtgcacagcaacacaaacacatacctggagtggtatctgcagaagcccggccagtctcctcagctgctgatctacaaggtgtccaacagattcagcggcgtgcccgacagattctctggctctggatctggcaccgacttcaccctgaagatctccagagtggaagccgaggacgtgggcgtgtacttctgtctccaggtcacacacgtgcccctgacatttggccagggcaccaagctggaaatcaag

SEQ ID NO: 95 - protein, 16 aa, Homo sapiens
RSSQSIVHSNTNTYLE

SEQ ID NO: 96 - protein, 112 aa, Homo sapiens
DVVMTQSPLSLPVTPGEPASISCRSSQSIVHSNANTYLEWYLQKPGQSPQLLIYKVSNRFSGVPDRFSGSGSGTDFTLKISRVEAEDVGVYFCLQVTHVPLTFGQGTKLEIK

SEQ ID NO: 97 - DNA, 336 bp, Homo sapiens
gacgtggtcatgacacagagccctctgagcctgcctgtgacacctggcgaacctgccagcatcagctgtagaagcagccagagcatcgtgcacagcaacgccaacacatacctggagtggtatctgcagaagcccggccagtctcctcagctgctgatctacaaggtgtccaacagattcagcggcgtgcccgacagattctctggctctggatctggcaccgacttcaccctgaagatctccagagtggaagccgaggacgtgggcgtgtacttctgtctccaggtcacacacgtgcccctgacatttggccagggcaccaagctggaaatcaag

SEQ ID NO: 98 - protein, 16 aa, Homo sapiens
RSSQSIVHSNANTYLE

SEQ ID NO: 99 - protein, 115 aa, Homo sapiens
QVQLVQSGAEVKKPGSSVKVSCKASGYTFADYEIHWVRQAPGQGLEWMGAIHPGSGGTAYNQKFQGRVTLTADKSSTTAYMELSSLRSEDTAVYYCTRYYSFAYWGQGTLVTVSS

SEQ ID NO: 100 - DNA, 345 bp, Homo sapiens
caggttcagctggttcagtctggcgccgaagtgaagaaacctggcagcagcgtgaaggtgtcctgcaaggctagcggctacaccttcgccgactacgagatccactgggtccgacaggctccaggacagggacttgaatggatgggcgctatccatcctggctctggcggcacagcttacaaccagaaattccagggcagagtgaccctgaccgccgacaagtctagcaccaccgcctacatggaactgagcagcctgagaagcgaggacaccgccgtgtactactgcacccggtactacagcttcgcctactggggacagggaaccctggtcacagtcagctct

SEQ ID NO: 101 - protein, 17 aa, Homo sapiens
AIHPGSGGTAYNQKFQG

SEQ ID NO: 102 - protein, 115 aa, Homo sapiens
QVQLVQSGAELKKPGSSVKVSCKASGYTFADYEIHWVRQAPGQGLEWMGAIHPGSGGTAYNQKFQGRVTLTADKSSTTAYMELSSLRSEDTAVYYCTRYYSFAYWGQGTLVTVSS

SEQ ID NO: 103 - DNA, 345 bp, Homo sapiens
caggttcagctggttcagtctggcgccgaactgaagaaacctggcagcagcgtgaaggtgtcctgcaaggctagcggctacaccttcgccgactacgagatccactgggtccgacaggctccaggacagggacttgaatggatgggcgctatccatcctggctctggcggcacagcttacaaccagaaattccagggcagagtgaccctgaccgccgacaagtctagcaccaccgcctacatggaactgagcagcctgagaagcgaggacaccgccgtgtactactgcacccggtactacagcttcgcctactggggacagggaaccctggtcacagtcagctct

SEQ ID NO: 104 - protein, 115 aa, Homo sapiens
QVQLVQSGAEVKKPGSSVKVSCKASGYTFADYEIHWVRQAPGQGLEWMGAIHPGSGGTAYAQKFQGRVTLTADKSSTTAYMELSSLRSEDTAVYYCTRYYSFAYWGQGTLVTVSS

SEQ ID NO: 105 - DNA, 345 bp, Homo sapiens
caggttcagctggttcagtctggcgccgaagtgaagaaacctggcagcagcgtgaaggtgtcctgcaaggctagcggctacaccttcgccgactacgagatccactgggtccgacaggctccaggacagggacttgaatggatgggcgctatccatcctggctctggcggcacagcttacgcccagaaattccagggcagagtgaccctgaccgccgacaagtctagcaccaccgcctacatggaactgagcagcctgagaagcgaggacaccgccgtgtactactgcacccggtactacagcttcgcctactggggacagggaaccctggtcacagtcagctct

SEQ ID NO: 106 - protein, 17 aa, Homo sapiens
AIHPGSGGTAYAQKFQG

SEQ ID NO: 107 - protein, 115 aa, Homo sapiens
QVQLVQSGAEVKKPGSSVKVSCKASGYTFADYEIHWVRQAPGQGLEWMGAIHPGSGGTAYNQKFQGRVTLTADESSTTAYMELSSLRSEDTAVYYCTRYYSFAYWGQGTLVTVSS

SEQ ID NO: 108 - DNA, 345 bp, Homo sapiens
caggttcagctggttcagtctggcgccgaagtgaagaaacctggcagcagcgtgaaggtgtcctgcaaggctagcggctacaccttcgccgactacgagatccactgggtccgacaggctccaggacagggacttgaatggatgggcgctatccatcctggctctggcggcacagcttacaaccagaaattccagggcagagtgaccctgaccgccgacgagtctagcaccaccgcctacatggaactgagcagcctgagaagcgaggacaccgccgtgtactactgcacccggtactacagcttcgcctactggggacagggaaccctggtcacagtcagctct

SEQ ID NO: 109 - protein, 115 aa, Homo sapiens
QVQLVQSGAELKKPGSSVKVSCKASGYTFADYEIHWVRQAPGQGLEWMGAIHPGSGGTAYNQKFQGRVTLTADESSTTAYMELSSLRSEDTAVYYCTRYYSFAYWGQGTLVTVSS

SEQ ID NO: 110 - DNA, 345 bp, Homo sapiens
caggttcagctggttcagtctggcgccgaactgaagaaacctggcagcagcgtgaaggtgtcctgcaaggctagcggctacaccttcgccgactacgagatccactgggtccgacaggctccaggacagggacttgaatggatgggcgctatccatcctggctctggcggcacagcttacaaccagaaattccagggcagagtgaccctgaccgccgacgagtctagcaccaccgcctacatggaactgagcagcctgagaagcgaggacaccgccgtgtactactgcacccggtactacagcttcgcctactggggacagggaaccctggtcacagtcagctct

SEQ ID NO: 111 - protein, 115 aa, Homo sapiens
QVQLVQSGAEVKKPGSSVKVSCKASGYTFADYEIHWVRQAPGQGLEWMGAIHPGSGGTAYAQKFQGRVTLTADESSTTAYMELSSLRSEDTAVYYCTRYYSFAYWGQGTLVTVSS

SEQ ID NO: 112 - DNA, 345 bp, Homo sapiens
caggttcagctggttcagtctggcgccgaagtgaagaaacctggcagcagcgtgaaggtgtcctgcaaggctagcggctacaccttcgccgactacgagatccactgggtccgacaggctccaggacagggacttgaatggatgggcgctatccatcctggctctggcggcacagcttacgcccagaaattccagggcagagtgaccctgaccgccgacgagtctagcaccaccgcctacatggaactgagcagcctgagaagcgaggacaccgccgtgtactactgcacccggtactacagcttcgcctactggggacagggaaccctggtcacagtcagctct

SEQ ID NO: 113 - protein, 109 aa, Homo sapiens
QAVVTQEPSLTVSPGGTVTLTCRSSTGAVTTSNYANWVQQKPGQAPRGLIGGTNKRAPWTPARFSGSLLGGKAALTLSGAQPEDEAEYYCALWYSNLWVFGGGTKLTVL

SEQ ID NO: 114 - DNA, 327 bp, Homo sapiens
caggctgtggtcacacaagagcctagcctgacagtgtctcctggcggcacagtgaccctgacctgtagatcttctacaggcgccgtgaccaccagcaactacgctaattgggtgcagcagaagcccggccaggctcctagaggactgatcggcggaacaaacaagagagccccttggacacccgccagattctctggatctctgctcggcggaaaggccgctctgacactttctggtgctcagcctgaggacgaggccgagtactattgtgccctgtggtacagcaacctgtgggtgttcggcggaggcaccaaactgacagttctg

SEQ ID NO: 115 - protein, 14 aa, Homo sapiens
RSSTGAVTTSNYAN

SEQ ID NO: 116 - protein, 8 aa, Homo sapiens
GGTNKRAP

SEQ ID NO: 117 - protein, 9 aa, Homo sapiens
ALWYSNLWV

SEQ ID NO: 118 - protein, 109 aa, Homo sapiens
QAVVTQEPSLTVSPGGTVTLTCRSSTGAVTTSNYANWVQEKPGQAPRGLIGGTNKRAPWTPARFSGSLLGGKAALTLSGAQPEDEAEYYCALWYSNLWVFGGGTKLTVL

SEQ ID NO: 119 - DNA, 327 bp, Homo sapiens
caggctgtggtcacacaagagcctagcctgacagtgtctcctggcggcacagtgaccctgacctgtagatcttctacaggcgccgtgaccaccagcaactacgctaattgggtgcaggagaagcccggccaggctcctagaggactgatcggcggaacaaacaagagagccccttggacacccgccagattctctggatctctgctcggcggaaaggccgctctgacactttctggtgctcagcctgaggacgaggccgagtactattgtgccctgtggtacagcaacctgtgggtgttcggcggaggcaccaaactgacagttctg

SEQ ID NO: 120 - protein, 109 aa, Homo sapiens
EAVVTQEPSLTVSPGGTVTLTCESSDGAVTTSNYANWVQEKPGQAPRGLIGGTNKEAPWTPARFSGSLLGGKAALTLSGAQPEDEAEYYCALWYSNLWVFGGGTKLTVL

SEQ ID NO: 121 - DNA, 327 bp, Homo sapiens
gaggctgtggtcacacaagagcctagcctgacagtgtctcctggcggcacagtgaccctgacctgtgagtcttctgacggcgccgtgaccaccagcaactacgctaattgggtgcaggagaagcccggccaggctcctagaggactgatcggcggaacaaacaaggaggccccttggacacccgccagattctctggatctctgctcggcggaaaggccgctctgacactttctggtgctcagcctgaggacgaggccgagtactattgtgccctgtggtacagcaacctgtgggtgttcggcggaggcaccaaactgacagttctg

SEQ ID NO: 122 - protein, 14 aa, Homo sapiens
ESSDGAVTTSNYAN

SEQ ID NO: 123 - protein, 8 aa, Homo sapiens
GGTNKEAP

SEQ ID NO: 124 - protein, 109 aa, Homo sapiens
QAVVTQEPSLTVSPGGTVTLTCESSDGAVTTSNYANWVQEKPGQAPRGLIGGTNKEAPWTPARFSGSLLGGKAALTLSGAQPEDEAEYYCALWYSNLWVFGGGTKLTVL

SEQ ID NO: 125 - DNA, 327 bp, Homo sapiens
caggctgtggtcacacaagagcctagcctgacagtgtctcctggcggcacagtgaccctgacctgtgagtcttctgacggcgccgtgaccaccagcaactacgctaattgggtgcaggagaagcccggccaggctcctagaggactgatcggcggaacaaacaaggaggccccttggacacccgccagattctctggatctctgctcggcggaaaggccgctctgacactttctggtgctcagcctgaggacgaggccgagtactattgtgccctgtggtacagcaacctgtgggtgttcggcggaggcaccaaactgacagttctg

SEQ ID NO: 126 - protein, 109 aa, Homo sapiens
QAVVTQEPSLTVSPGGTVTLTCRSSTGAVTTSNYANWVQEKPGQAPRGLIGGTNKRAPWTPARFSGSLLGGKAALTITGAQAEDEAEYYCVLWYSNLWVFGGGTKLTVL

SEQ ID NO: 127 - DNA, 327 bp, Homo sapiens
caggctgtggtcacacaagagcctagcctgacagtgtctcctggcggcacagtgaccctgacctgtagatcttctacaggcgccgtgaccaccagcaactacgctaattgggtgcaggagaagcccggccaggctcctagaggactgatcggcggaacaaacaagagagccccttggacacccgccagattctctggatctctgctcggcggaaaggccgctctgacaatcactggtgctcaggctgaggacgaggccgagtactattgtgtgctgtggtacagcaacctgtgggtgttcggcggaggcaccaaactgacagttctg

SEQ ID NO: 128 - protein, 9 aa, Homo sapiens
VLWYSNLWV

SEQ ID NO: 129 - protein, 109 aa, Homo sapiens
QAVVTQEPSLTVSPGGTVTLTCRSSTGAVTTSNYANWFQEKPGQAPRGLIYGTNKRAPWTPARFSGSLLGGKAALTLSGAQAEDEAEYYCVLWYSNLWVFGGGTKLTVL

SEQ ID NO: 130 - DNA, 327 bp, Homo sapiens
caggctgtggtcacacaagagcctagcctgacagtgtctcctggcggcacagtgaccctgacctgtagatcttctacaggcgccgtgaccaccagcaactacgctaattggttccaggagaagcccggccaggctcctagaggactgatctacggaacaaacaagagagccccttggacacccgccagattctctggatctctgctcggcggaaaggccgctctgacactttctggtgctcaggctgaggacgaggccgagtactattgtgtcctgtggtacagcaacctgtgggtgttcggcggaggcaccaaactgacagttctg

SEQ ID NO: 131 - protein, 8 aa, Homo sapiens
YGTNKRAP

SEQ ID NO: 132 - protein, 125 aa, Homo sapiens
EVQLVESGGGLVQPGGSLRLSCAASGFTFNTYAMNWVRQAPGKGLEWVSRIRSKYNNYATYYADSVKDRFTISRDDSKNTLYLQMNSLRAEDTAVYYCVRHGNFGNSYVSWFAYWGQGTLVTVSS

SEQ ID NO: 133 - DNA, 375 bp, Homo sapiens
gaggtgcagctggttgaatctggcggaggactggttcagcctggcggatctctgagactgtcttgtgccgccagcggcttcaccttcaacacctacgctatgaactgggtccgacaggcccctggcaaaggactggaatgggtgtccagaatcaggtccaagtacaacaactacgccacctactacgccgacagcgtgaaggacagattcaccatcagcagggacgacagcaagaacaccctgtacctgcagatgaacagcctgagagccgaggacaccgccgtgtactactgtgtcagacacggcaacttcggcaacagctatgtgtcttggtttgcctactggggccagggcacactggtcacagttagctct

SEQ ID NO: 134 - protein, 6 aa, Homo sapiens
NTYAMN

SEQ ID NO: 135 - protein, 18 aa, Homo sapiens
IRSKYNNYATYYADSVKD

SEQ ID NO: 136 - protein, 14 aa, Homo sapiens
HGNFGNSYVSWFAY

SEQ ID NO: 137 - protein, 125 aa, Homo sapiens
EVQLVESGGGLVQPGGSLRLSCAASGFTFSTYAMNWVRKAPGKGLEWVSRIRSKYNNYATYYADSVKDRFTISRDDSKNTLYLQMNSLRAEDTAVYYCVRHGNFGNSYVSWFAYWGQGTLVTVSS

SEQ ID NO: 138 - DNA, 375 bp, Homo sapiens
gaggtgcagctggttgaatctggcggaggactggttcagcctggcggatctctgagactgtcttgtgccgccagcggcttcaccttctccacctacgctatgaactgggtccgaaaggcccctggcaaaggactggaatgggtgtccagaatcaggtccaagtacaacaactacgccacctactacgccgacagcgtgaaggacagattcaccatcagcagggacgacagcaagaacaccctgtacctgcagatgaacagcctgagagccgaggacaccgccgtgtactactgtgtcagacacggcaacttcggcaacagctatgtgtcttggtttgcctactggggccagggcacactggtcacagttagctct

SEQ ID NO: 139 - protein, 6 aa, Homo sapiens
STYAMN

SEQ ID NO: 140 - protein, 125 aa, Homo sapiens
EVQLVESGGGLVQPGGSLRLSCAASGFTFSTYAMNWVRKAPGKGLEWVSRIRSKYNNYATYYADSVKDRFTISRDDSKNTLYLQMNSLRAEDTAVYYCVRHGNFGESYVSWFAYWGQGTLVTVSS

SEQ ID NO: 141 - DNA, 375 bp, Homo sapiens
gaggtgcagctggttgaatctggcggaggactggttcagcctggcggatctctgagactgtcttgtgccgccagcggcttcaccttctccacctacgctatgaactgggtccgaaaggcccctggcaaaggactggaatgggtgtccagaatcaggtccaagtacaacaactacgccacctactacgccgacagcgtgaaggacagattcaccatcagcagggacgacagcaagaacaccctgtacctgcagatgaacagcctgagagccgaggacaccgccgtgtactactgtgtcagacacggcaacttcggcgagagctatgtgtcttggtttgcctactggggccagggcacactggtcacagttagctct

SEQ ID NO: 142 - protein, 14 aa, Homo sapiens
HGNFGESYVSWFAY

SEQ ID NO: 143 - protein, 125 aa, Homo sapiens
EVQLVESGGGLVQPGGSLRLSCAASGFTFSTYAMNWVRKAPGKGLEWVSRIRSKYNNYATYYADSVKDRFTISRDDSKNTLYLQMNSLRAEDTAVYYCVRHGNFGQSYVSWFAYWGQGTLVTVSS

SEQ ID NO: 144 - DNA, 375 bp, Homo sapiens
gaggtgcagctggttgaatctggcggaggactggttcagcctggcggatctctgagactgtcttgtgccgccagcggcttcaccttctccacctacgctatgaactgggtccgaaaggcccctggcaaaggactggaatgggtgtccagaatcaggtccaagtacaacaactacgccacctactacgccgacagcgtgaaggacagattcaccatcagcagggacgacagcaagaacaccctgtacctgcagatgaacagcctgagagccgaggacaccgccgtgtactactgtgtcagacacggcaacttcggccagagctatgtgtcttggtttgcctactggggccagggcacactggtcacagttagctct

SEQ ID NO: 145 - protein, 14 aa, Homo sapiens
HGNFGQSYVSWFAY

SEQ ID NO: 146 - protein, 125 aa, Homo sapiens
EVQLVESGGGLVQPGGSLRLSCAASGFTFSTYAMNWVRKAPGKGLEWVSRIRSKYNNYATYYADSVKDRFTISRDDSKNTLYLQMNSLRAEDTAVYYCVRHGNFGDSYVSWFAYWGQGTLVTVSS

SEQ ID NO: 147 - DNA, 375 bp, Homo sapiens
gaggtgcagctggttgaatctggcggaggactggttcagcctggcggatctctgagactgtcttgtgccgccagcggcttcaccttctccacctacgctatgaactgggtccgaaaggcccctggcaaaggactggaatgggtgtccagaatcaggtccaagtacaacaactacgccacctactacgccgacagcgtgaaggacagattcaccatcagcagggacgacagcaagaacaccctgtacctgcagatgaacagcctgagagccgaggacaccgccgtgtactactgtgtcagacacggcaacttcggcgacagctatgtgtcttggtttgcctactggggccagggcacactggtcacagttagctct

SEQ ID NO: 148 - protein, 14 aa, Homo sapiens
HGNFGDSYVSWFAY

SEQ ID NO: 149 - protein, 125 aa, Homo sapiens
EVQLVESGGGLVQPGGSLRLSCAASGFTFSTYAMNWVRKAPGKGLEWVSRIRSKYNNYATYYADSVKDRFTISRDDSKNTLYLQMNSLRAEDTAVYYCVRHGNFGTSYVSWFAYWGQGTLVTVSS

SEQ ID NO: 150 - DNA, 375 bp, Homo sapiens
gaggtgcagctggttgaatctggcggaggactggttcagcctggcggatctctgagactgtcttgtgccgccagcggcttcaccttctccacctacgctatgaactgggtccgaaaggcccctggcaaaggactggaatgggtgtccagaatcaggtccaagtacaacaactacgccacctactacgccgacagcgtgaaggacagattcaccatcagcagggacgacagcaagaacaccctgtacctgcagatgaacagcctgagagccgaggacaccgccgtgtactactgtgtcagacacggcaacttcggcaccagctatgtgtcttggtttgcctactggggccagggcacactggtcacagttagctct

SEQ ID NO: 151 - protein, 14 aa, Homo sapiens
HGNFGTSYVSWFAY

SEQ ID NO: 152 - protein, 125 aa, Homo sapiens
EVQLVESGGGLVQPGGSLRLSCAASGFTFSDYAMNWVRKAPGKGLEWVSRIRSKYNNYATYYADSVEDRFTISRDDSKNTLYLQMNSLRAEDTAVYYCVRHGNFGNSYVSWFAYWGQGTLVTVSS

SEQ ID NO: 153 - DNA, 375 bp, Homo sapiens
gaggtgcagctggttgaatctggcggaggactggttcagcctggcggatctctgagactgtcttgtgccgccagcggcttcaccttctccgactacgctatgaactgggtccgaaaggcccctggcaaaggactggaatgggtgtccagaatcaggtccaagtacaacaactacgccacctactacgccgacagcgtggaggacagattcaccatcagcagggacgacagcaagaacaccctgtacctgcagatgaacagcctgagagccgaggacaccgccgtgtactactgtgtcagacacggcaacttcggcaacagctatgtgtcttggtttgcctactggggccagggcacactggtcacagttagctct

SEQ ID NO: 154 - protein, 6 aa, Homo sapiens
SDYAMN

SEQ ID NO: 155 - protein, 18 aa, Homo sapiens
IRSKYNNYATYYADSVED

SEQ ID NO: 156 - protein, 125 aa, Homo sapiens
EVQLVESGGGLVQPGGSLRLSCAASGFTFNTYAMNWVRKAPGKGLEWVGRIRSKYNNYATYYADSVKDRFTISRDDSKNSLYLQMNSLKTEDTAVYYCARHGNFGNSYVSWFAYWGQGTLVTVSS

SEQ ID NO: 157 - DNA, 375 bp, Homo sapiens
gaggtgcagctggttgaatctggcggaggactggttcagcctggcggatctctgagactgtcttgtgccgccagcggcttcaccttcaacacctacgctatgaactgggtccgaaaggcccctggcaaaggactggaatgggtgggaagaatcaggtccaagtacaacaactacgccacctactacgccgacagcgtgaaggacagattcaccatcagcagggacgacagcaagaacagcctgtacctgcagatgaacagcctgaaaaccgaggacaccgccgtgtactactgtgccagacacggcaacttcggcaacagctatgtgtcttggtttgcctactggggccagggcacactggtcacagttagctct

SEQ ID NO: 158 - protein, 125 aa, Homo sapiens
EVQLVESGGGLVQPGGSLRLSCAASGFTFNTYAMNWVRKAPGKGLEWVGRIRSKYNNYATYYADSVKDRFTISRDDSKNSLYLQMNSLKTEDTAVYYCVRHGNFGNSYVSWFAYWGQGTLVTVSS

SEQ ID NO: 159 - DNA, 375 bp, Homo sapiens
gaggtgcagctggttgaatctggcggaggactggttcagcctggcggatctctgagactgtcttgtgccgccagcggcttcaccttcaacacctacgctatgaactgggtccgaaaggcccctggcaaaggactggaatgggtgggaagaatcaggtccaagtacaacaactacgccacctactacgccgacagcgtgaaggacagattcaccatcagcagggacgacagcaagaacagcctgtacctgcagatgaacagcctgaaaaccgaggacaccgccgtgtactactgtgtcagacacggcaacttcggcaacagctatgtgtcttggtttgcctactggggccagggcacactggtcacagttagctct

SEQ ID NO: 160 - protein, 125 aa, Homo sapiens
EVQLVESGGGLVQPGGSLRLSCAASGFTFNTYAMNWVRKAPGKGLEWVARIRSKYNNYATYYADSVKDRFTISRDDSKNSLYLQMNSLKTEDTAVYYCVRHGNFGNSYVSWFAYWGQGTLVTVSS

SEQ ID NO: 161 - DNA, 375 bp, Homo sapiens
gaggtgcagctggttgaatctggcggaggactggttcagcctggcggatctctgagactgtcttgtgccgccagcggcttcaccttcaacacctacgctatgaactgggtccgaaaggcccctggcaaaggactggaatgggtggccagaatcaggtccaagtacaacaactacgccacctactacgccgacagcgtgaaggacagattcaccatcagcagggacgacagcaagaacagcctgtacctgcagatgaacagcctgaaaaccgaggacaccgccgtgtactactgtgtcagacacggcaacttcggcaacagctatgtgtcttggtttgcctactggggccagggcacactggtcacagttagctct

SEQ ID NO: 162 - protein, 219 aa, Homo sapiens
DVVMTQSPLSLPVTPGEPASISCRSSQSIVHSNGNTYLEWYLKKPGQSPQLLIYKVSNRFSGVPDRFSGSGSGTDFTLKISRVEAEDVGVYFCLQVTHVPLTFGQGTKLEIKRTVAAPSVFIFPPSDEQLKSGTASVVCLLNNFYPREAKVQWKVDNALQSGNSQESVTEQDSKDSTYSLSSTLTLSKADYEKHKVYACEVTHQGLSSPVTKSFNRGEC

SEQ ID NO: 163 - DNA, 657 bp, Homo sapiens
gacgtggtcatgacacagagccctctgagcctgcctgtgacacctggcgaacctgccagcatcagctgtagaagcagccagagcatcgtgcacagcaacggcaacacatacctggagtggtatctgaagaagcccggccagtctcctcagctgctgatctacaaggtgtccaacagattcagcggcgtgcccgacagattctctggctctggatctggcaccgacttcaccctgaagatctccagagtggaagccgaggacgtgggcgtgtacttctgtctccaggtcacacacgtgcccctgacatttggccagggcaccaagctggaaatcaagcgaactgtggctgcaccatctgtcttcatcttcccgccatctgatgagcagttgaaatctggaactgcctctgttgtgtgcctgctgaataacttctatcccagagaggccaaagtacagtggaaggtggataacgccctccaatcgggtaactcccaggagagtgtcacagagcaggacagcaaggacagcacctacagcctcagcagcaccctgacgctgagcaaagcagactacgagaaacacaaagtctacgcctgcgaagtcacccatcagggcctgagctcgcccgtcacaaagagcttcaacaggggagagtgt

SEQ ID NO: 164 - protein, 442 aa, Homo sapiens
QVQLVQSGAEVKKPGSSVKVSCKASGYTFADYEIHWVREAPGQGLEWMGAIHPGSGGTAYAQKFQGRVTLTADESSTTAYMELSSLRSEDTAVYYCTRYYSFAYWGQGTLVTVSSASTKGPSVFPLAPCSRSTSESTAALGCLVKDYFPEPVTVSWNSGALTSGVHTFPAVLQSSGLYSLSSVVTVPSSSLGTKTYTCNVDHKPSNTKVDKRVESKYGPPCPPCPAPEFEGGPSVFLFPPKPKDTLMISRTPEVTCVVVDVSQEDPEVQFNWYVDGVEVHNAKTKPREEQFNSTYRVVSVLTVLHQDWLNGKEYKCKVSNKGLASSIEKTISKAKGQPREPQVCTLPPSQEEMTKNQVSLSCAVKGFYPSDIAVEWESNGQPENNYKTTPPVLDSDGSFFLVSKLTVDKSRWQEGNVFSCSVMHEALHNHYTQKSLSLSLGK

SEQ ID NO: 165 - DNA, 1326 bp, Homo sapiens
caggttcagctggttcagtctggcgccgaagtgaagaaacctggcagcagcgtgaaggtgtcctgcaaggctagcggctacaccttcgccgactacgagatccactgggtccgagaggctccaggacagggacttgaatggatgggcgctatccatcctggctctggcggcacagcttacgcccagaaattccagggcagagtgaccctgaccgccgacgagtctagcaccaccgcctacatggaactgagcagcctgagaagcgaggacaccgccgtgtactactgcacccggtactacagcttcgcctactggggacagggaaccctggtcacagtcagctctgctagcaccaagggccccagcgtgttccccctggccccttgcagcagaagcaccagcgagagcacagccgccctgggctgcctggtgaaggactacttccccgagcccgtgaccgtgtcctggaacagcggcgctctgaccagcggcgtgcataccttccccgccgtgctccagagcagcggactgtactccctgagcagcgtggtgaccgtgccttccagcagcctgggcaccaagacctacacctgcaacgtggaccacaagcccagcaacaccaaggtggacaagagagtggagagcaagtacggccctccctgccccccttgccctgcccccgagttcgagggcggacctagcgtgttcctgttcccccccaagcccaaggacaccctgatgatcagcagaacccccgaggtgacctgcgtggtggtggacgtgtcccaggaggaccccgaggtccagtttaattggtacgtggacggcgtggaagtgcataacgccaagaccaagcccagagaggagcagttcaacagcacctacagagtggtgtccgtgctgaccgtgctgcaccaggactggctgaacggcaaggaatacaagtgcaaggtctccaacaagggcctggccagcagcatcgagaagaccatcagcaaggccaagggccagccacgggagccccaggtctgcaccctgccacctagccaagaggagatgaccaagaaccaggtgtccctgagctgtgccgtgaaaggcttctatcccagcgatatcgccgtggagtgggagagcaacggccagcccgagaacaactacaagaccaccccccctgtgctggacagcgacggcagcttcttcctggtttccaagctgaccgtggacaagtccagatggcaggagggcaacgtcttcagctgctccgtgatgcacgaggccctgcacaaccactacacccagaagtccctgagcctgagcctgggcaag

SEQ ID NO: 166 - protein, 215 aa, Homo sapiens
QAVVTQEPSLTVSPGGTVTLTCRSSTGAVTTSNYANWVQEKPGQAPRGLIGGTNKRAPWTPARFSGSLLGGKAALTITGAQAEDEAEYYCVLWYSNLWVFGGGTKLTVLGQPKAAPSVTLFPPSSEELQANKATLVCLISDFYPGAVTVAWKADSSPVKAGVETTTPSKQSNNKYAASSYLSLTPEQWKSHRSYSCQVTHEGSTVEKTVAPTECS

SEQ ID NO: 167 - DNA, 645 bp, Homo sapiens
caggctgtggtcacacaagagcctagcctgacagtgtctcctggcggcacagtgaccctgacctgtagatcttctacaggcgccgtgaccaccagcaactacgctaattgggtgcaggagaagcccggccaggctcctagaggactgatcggcggaacaaacaagagagccccttggacacccgccagattctctggatctctgctcggcggaaaggccgctctgacaatcactggtgctcaggctgaggacgaggccgagtactattgtgtgctgtggtacagcaacctgtgggtgttcggcggaggcaccaaactgacagttctgggtcagcccaaggcggcgccctcggtcactctgttcccgccctcctctgaggagcttcaagccaacaaggccacactggtgtgtctcataagtgacttctatccgggagccgtgacagtggcctggaaggcagatagcagccccgtcaaggcgggagtggagaccaccacaccctccaaacaaagcaacaacaagtacgcggccagcagctacctgagcctgacgcctgagcagtggaagtcccacagaagctacagctgccaggtcacgcatgaagggagcaccgtggagaagacagtggcccctacagaatgttca

SEQ ID NO: 168 - protein, 452 aa, Homo sapiens
EVQLVESGGGLVQPGGSLRLSCAASGFTFNTYAMNWVRKAPGKGLEWVGRIRSKYNNYATYYADSVKDRFTISRDDSKNSLYLQMNSLKTEDTAVYYCVRHGNFGNSYVSWFAYWGQGTLVTVSSASTKGPSVFPLAPCSRSTSESTAALGCLVKDYFPEPVTVSWNSGALTSGVHTFPAVLQSSGLYSLSSVVTVPSSSLGTKTYTCNVDHKPSNTKVDKRVESKYGPPCPPCPAPEFEGGPSVFLFPPKPKDTLMISRTPEVTCVVVDVSQEDPEVQFNWYVDGVEVHNAKTKPREEQFNSTYRVVSVLTVLHQDWLNGKEYKCKVSNKGLASSIEKTISKAKGQPREPQVYTLPPCQEEMTKNQVSLWCLVKGFYPSDIAVEWESNGQPENNYKTTPPVLDSDGSFFLYSKLTVDKSRWQEGNVFSCSVMHEALHNHYTQKSLSLSLGK

SEQ ID NO: 169 - DNA, 1356 bp, Homo sapiens
gaggtgcagctggttgaatctggcggaggactggttcagcctggcggatctctgagactgtcttgtgccgccagcggcttcaccttcaacacctacgctatgaactgggtccgaaaggcccctggcaaaggactggaatgggtgggaagaatcaggtccaagtacaacaactacgccacctactacgccgacagcgtgaaggacagattcaccatcagcagggacgacagcaagaacagcctgtacctgcagatgaacagcctgaaaaccgaggacaccgccgtgtactactgtgtcagacacggcaacttcggcaacagctatgtgtcttggtttgcctactggggccagggcacactggtcacagttagctctgctagcaccaagggccccagcgtgttccccctggccccttgcagcagaagcaccagcgagagcacagccgccctgggctgcctggtgaaggactacttccccgagcccgtgaccgtgtcctggaacagcggcgctctgaccagcggcgtgcataccttccccgccgtgctccagagcagcggactgtactccctgagcagcgtggtgaccgtgccttccagcagcctgggcaccaagacctacacctgcaacgtggaccacaagcccagcaacaccaaggtggacaagagagtggagagcaagtacggccctccctgccccccttgccctgcccccgagttcgagggcggacctagcgtgttcctgttcccccccaagcccaaggacaccctgatgatcagcagaacccccgaggtgacctgcgtggtggtggacgtgtcccaggaggaccccgaggtccagtttaattggtacgtggacggcgtggaagtgcataacgccaagaccaagcccagagaggagcagttcaacagcacctacagagtggtgtccgtgctgaccgtgctgcaccaggactggctgaacggcaaggaatacaagtgcaaggtctccaacaagggcctggccagcagcatcgagaagaccatcagcaaggccaagggccagccacgggagccccaggtctacaccctgccaccttgtcaagaggagatgaccaagaaccaggtgtccctgtggtgtctggtgaaaggcttctatcccagcgatatcgccgtggagtgggagagcaacggccagcccgagaacaactacaagaccaccccccctgtgctggacagcgacggcagcttcttcctgtactccaagctgaccgtggacaagtccagatggcaggagggcaacgtcttcagctgctccgtgatgcacgaggccctgcacaaccactacacccagaagtccctgagcctgagcctgggcaag

SEQ ID NO: 170 - protein, 219 aa, Homo sapiens
DVVMTQSPLSLPVTPGEPASISCRSSQSIVHSNGNTYLEWYLKKPGQSPQLLIYKVSNRFSGVPDRFSGSGSGTDFTLKISRVEAEDVGVYFCLQVTHVPLTFGQGTKLEIKRTVAAPSVFIFPPSDKKLKSGTASVVCLLNNFYPREAKVQWKVDNALQSGNSQESVTEQDSKDSTYSLSSTLTLSKADYEKHKVYACEVTHQGLSSPVTKSFNRGEC

SEQ ID NO: 171 - DNA, 657 bp, Homo sapiens
gacgtggtcatgacacagagccctctgagcctgcctgtgacacctggcgaacctgccagcatcagctgtagaagcagccagagcatcgtgcacagcaacggcaacacatacctggagtggtatctgaagaagcccggccagtctcctcagctgctgatctacaaggtgtccaacagattcagcggcgtgcccgacagattctctggctctggatctggcaccgacttcaccctgaagatctccagagtggaagccgaggacgtgggcgtgtacttctgtctccaggtcacacacgtgcccctgacatttggccagggcaccaagctggaaatcaagcgaactgtggctgcaccatctgtcttcatcttcccgccatctgataagaaattgaaatctggaactgcctctgttgtgtgcctgctgaataacttctatcccagagaggccaaagtacagtggaaggtggataacgccctccaatcgggtaactcccaggagagtgtcacagagcaggacagcaaggacagcacctacagcctcagcagcaccctgacgctgagcaaagcagactacgagaaacacaaagtctacgcctgcgaagtcacccatcagggcctgagctcgcccgtcacaaagagcttcaacaggggagagtgt

SEQ ID NO: 172 - protein, 442 aa, Homo sapiens
QVQLVQSGAEVKKPGSSVKVSCKASGYTFADYEIHWVREAPGQGLEWMGAIHPGSGGTAYAQKFQGRVTLTADESSTTAYMELSSLRSEDTAVYYCTRYYSFAYWGQGTLVTVSSASTKGPSVFPLAPCSRSTSESTAALGCLVEDYFPEPVTVSWNSGALTSGVHTFPAVLQSSGLYSLSSVVTVPSSSLGTKTYTCNVDHKPSNTKVDERVESKYGPPCPPCPAPEFEGGPSVFLFPPKPKDTLMISRTPEVTCVVVDVSQEDPEVQFNWYVDGVEVHNAKTKPREEQFNSTYRVVSVLTVLHQDWLNGKEYKCKVSNKGLASSIEKTISKAKGQPREPQVCTLPPSQEEMTKNQVSLSCAVKGFYPSDIAVEWESNGQPENNYKTTPPVLDSDGSFFLVSKLTVDKSRWQEGNVFSCSVMHEALHNHYTQKSLSLSLGK

SEQ ID NO: 173 - DNA, 1326 bp, Homo sapiens
caggttcagctggttcagtctggcgccgaagtgaagaaacctggcagcagcgtgaaggtgtcctgcaaggctagcggctacaccttcgccgactacgagatccactgggtccgagaggctccaggacagggacttgaatggatgggcgctatccatcctggctctggcggcacagcttacgcccagaaattccagggcagagtgaccctgaccgccgacgagtctagcaccaccgcctacatggaactgagcagcctgagaagcgaggacaccgccgtgtactactgcacccggtactacagcttcgcctactggggacagggaaccctggtcacagtcagctctgctagcaccaagggccccagcgtgttccccctggccccttgcagcagaagcaccagcgagagcacagccgccctgggctgcctggtggaggactacttccccgagcccgtgaccgtgtcctggaacagcggcgctctgaccagcggcgtgcataccttccccgccgtgctccagagcagcggactgtactccctgagcagcgtggtgaccgtgccttccagcagcctgggcaccaagacctacacctgcaacgtggaccacaagcccagcaacaccaaggtggacgagagagtggagagcaagtacggccctccctgccccccttgccctgcccccgagttcgaaggcggacctagcgtgttcctgttcccccccaagcccaaggacaccctgatgatcagcagaacccccgaggtgacctgcgtggtggtggacgtgtcccaggaggaccccgaggtccagtttaattggtacgtggacggcgtggaagtgcataacgccaagaccaagcccagagaggagcagttcaacagcacctacagagtggtgtccgtgctgaccgtgctgcaccaggactggctgaacggcaaggaatacaagtgcaaggtctccaacaagggcctggccagcagcatcgagaagaccatcagcaaggccaagggccagccacgggagccccaggtctgcaccctgccacctagccaagaggagatgaccaagaaccaggtgtccctgagctgtgccgtgaaaggcttctatcccagcgatatcgccgtggagtgggagagcaacggccagcccgagaacaactacaagaccaccccccctgtgctggacagcgacggcagcttcttcctggtttccaagctgaccgtggacaagtccagatggcaggagggcaacgtcttcagctgctccgtgatgcacgaggccctgcacaaccactacacccagaagtccctgagcctgagcctgggcaag